European Patent Application EP 4 721 758 A1, published April 8, 2026. Title: Novel medicine for treating osteosarcoma. Applicant: 公益財団法人がん研究会. Application JP. The sequence listing filed with the application follows.

SEQUENCE LISTING (20 sequences)

SEQ ID NO: 1 - DNA, 20 bp, synthetic construct
  source 1..20: mol_type = other DNA
cttccaaggtaagggggttc

SEQ ID NO: 2 - DNA, 21 bp, synthetic construct
  source 1..21: mol_type = other DNA
actgactcgtttccggtttcc

SEQ ID NO: 3 - DNA, 20 bp, synthetic construct
  source 1..20: mol_type = other DNA
atgggacgtgtgttacctgc

SEQ ID NO: 4 - DNA, 20 bp, synthetic construct
  source 1..20: mol_type = other DNA
tagtccggggttccttctgt

SEQ ID NO: 5 - DNA, 20 bp, synthetic construct
  source 1..20: mol_type = other DNA
ttcttctgtgttcgtccgca

SEQ ID NO: 6 - DNA, 20 bp, synthetic construct
  source 1..20: mol_type = other DNA
gacaccaacaggaaagggct

SEQ ID NO: 7 - DNA, 20 bp, synthetic construct
  source 1..20: mol_type = other DNA
agggaggatgggtggtaact

SEQ ID NO: 8 - DNA, 20 bp, synthetic construct
  source 1..20: mol_type = other DNA
cgaatgttcttgccacctgc

SEQ ID NO: 9 - DNA, 20 bp, synthetic construct
  source 1..20: mol_type = other DNA
acccctattgccctttggtg

SEQ ID NO: 10 - DNA, 20 bp, synthetic construct
  source 1..20: mol_type = other DNA
ctgccatgcaagaaagcgtt

SEQ ID NO: 11 - DNA, 20 bp, synthetic construct
  source 1..20: mol_type = other DNA
cctctcccgacctgtgatac

SEQ ID NO: 12 - DNA, 20 bp, synthetic construct
  source 1..20: mol_type = other DNA
cttcctcggaaagtcactcc

SEQ ID NO: 13 - DNA, 20 bp, synthetic construct
  source 1..20: mol_type = other DNA
aaagccgctcaactacatgg

SEQ ID NO: 14 - DNA, 21 bp, synthetic construct
  source 1..21: mol_type = other DNA
tgctttgaatgcgtcccagag

SEQ ID NO: 15 - DNA, 20 bp, synthetic construct
  source 1..20: mol_type = other DNA
atccgccattctcatgcctt

SEQ ID NO: 16 - DNA, 20 bp, synthetic construct
  source 1..20: mol_type = other DNA
tttaacaaggcagggagggc

SEQ ID NO: 17 - DNA, 20 bp, synthetic construct
  source 1..20: mol_type = other DNA
ccttctttgagttcggtggg

SEQ ID NO: 18 - DNA, 20 bp, synthetic construct
  source 1..20: mol_type = other DNA
tcttcagagacagccaggag

SEQ ID NO: 19 - DNA, 19 bp, synthetic construct
  source 1..19: mol_type = other DNA
atggggaaggtgaaggtcg

SEQ ID NO: 20 - DNA, 22 bp, synthetic construct
  source 1..22: mol_type = other DNA
ggggtcattgatggcaacaata